European Patent Specification EP 3 356 826 B1, published December 6, 2023. Title: GDF-15 as a diagnostic marker for melanoma. Applicant: Julius-Maximilians-Universität Würzburg. The sequence listing filed with the application follows.

SEQUENCE LISTING (26 sequences)

SEQ ID NO: 1 - protein, 97 aa, Mus musculus
QVKLQQSGPGILQSSQTLSLTCSFSGFSLSTSGMGVSWIRQPSGKGLEWLAHIYWDDDKRYNPTLKSRLTISKDPSRNQVFLKITSVDTADTATYYC

SEQ ID NO: 2 - protein, 88 aa, Mus musculus
DIVLTQSPKFMSTSVGDRVSVTCKASQNVGTNVAWFLQKPGQSPKALIYSASYRYSGVPDRFTGSGSGTDFTLTISNVQSEDLAEYFC

SEQ ID NO: 3 - protein, 10 aa, Mus musculus
GFSLSTSGMG

SEQ ID NO: 4 - protein, 7 aa, Mus musculus
IYWDDDK

SEQ ID NO: 5 - protein, 10 aa, Mus musculus
ARSSYGAMDY

SEQ ID NO: 6 - protein, 6 aa, Mus musculus
QNVGTN

SEQ ID NO: 7 - protein, 9 aa, Mus musculus
QQYNNFPYT

SEQ ID NO: 8 - protein, 114 aa, Artificial Sequence
  recombinant mature human GDF-15 protein
GSARNGDHCPLGPGRCCRLHTVRASLEDLGWADWVLSPREVQVTMCIGACPSQFRAANMHAQIKTSLHRLKPDTVPAPCCVPASYNPMVLIQKTDTGVSLQTYDDLLAKDCHCI

SEQ ID NO: 9 - protein, 308 aa, Homo sapiens
MPGQELRTVNGSQMLLVLLVLSWLPHGGALSLAEASRASFPGPSELHSEDSRFRELRKRYEDLLTRLRANQSWEDSNTDLVPAPAVRILTPEVRLGSGGHLHLRISRAALPEGLPEASRLHRALFRLSPTASRSWDVTRPLRRQLSLARPQAPALHLRLSPPPSQSDQLLAESSSARPQLELHLRPQAARGRRRARARNGDHCPLGPGRCCRLHTVRASLEDLGWADWVLSPREVQVTMCIGACPSQFRAANMHAQIKTSLHRLKPDTVPAPCCVPASYNPMVLIQKTDTGVSLQTYDDLLAKDCHCI

SEQ ID NO: 10 - protein, 322 aa, Artificial Sequence
  human GDF-15 precursor protein + N-terminal and C-terminal GSGS linker
GSGSGSGMPGQELRTVNGSQMLLVLLVLSWLPHGGALSLAEASRASFPGPSELHSEDSRFRELRKRYEDLLTRLRANQSWEDSNTDLVPAPAVRILTPEVRLGSGGHLHLRISRAALPEGLPEASRLHRALFRLSPTASRSWDVTRPLRRQLSLARPQAPALHLRLSPPPSQSDQLLAESSSARPQLELHLRPQAARGRRRARARNGDHCPLGPGRCCRLHTVRASLEDLGWADWVLSPREVQVTMCIGACPSQFRAANMHAQIKTSLHRLKPDTVPAPCCVPASYNPMVLIQKTDTGVSLQTYDDLLAKDCHCIGSGSGSG

SEQ ID NO: 11 - protein, 10 aa, Artificial Sequence
  Flag peptide
DYKDDDDKGG

SEQ ID NO: 12 - protein, 10 aa, Artificial Sequence
  HA peptide
YPYDVPDYAG

SEQ ID NO: 13 - protein, 13 aa, Artificial Sequence
  peptide derived from human GDF-15
ELHLRPQAARGRR

SEQ ID NO: 14 - protein, 13 aa, Artificial Sequence
  peptide derived from human GDF-15
LHLRPQAARGRRR

SEQ ID NO: 15 - protein, 13 aa, Artificial Sequence
  peptide derived from human GDF-15
HLRPQAARGRRRA

SEQ ID NO: 16 - protein, 13 aa, Artificial Sequence
  peptide derived from human GDF-15
LRPQAARGRRRAR

SEQ ID NO: 17 - protein, 13 aa, Artificial Sequence
  peptide derived from human GDF-15
RPQAARGRRRARA

SEQ ID NO: 18 - protein, 13 aa, Artificial Sequence
  peptide derived from human GDF-15
PQAARGRRRARAR

SEQ ID NO: 19 - protein, 13 aa, Artificial Sequence
  peptide derived from human GDF-15
QAARGRRRARARN

SEQ ID NO: 20 - protein, 13 aa, Artificial Sequence
  peptide derived from human GDF-15
MHAQIKTSLHRLK

SEQ ID NO: 21 - DNA, 291 bp, Mus musculus
caagtgaagctgcagcagtcaggccctgggatattgcagtcctcccagaccctcagtctgacttgttctttctctgggttttcactgagtacttctggtatgggtgtgagctggattcgtcagccttcaggaaagggtctggagtggctggcacacatttactgggatgatgacaagcgctataacccaaccctgaagagccggctcacaatctccaaggatccctccagaaaccaggtattcctcaagatcaccagtgtggacactgcagatactgccacatactactgt

SEQ ID NO: 22 - DNA, 264 bp, Mus musculus
gacattgtgctcacccagtctccaaaattcatgtccacatcagtaggagacagggtcagcgtcacctgcaaggccagtcagaatgtgggtactaatgtggcctggtttctacagaaaccagggcaatctcctaaagcacttatttactcggcatcctaccggtacagtggagtccctgatcgcttcacaggcagtggatctgggacagatttcactctcaccatcagcaacgtgcagtctgaagacttggcagagtatttctgt

SEQ ID NO: 23 - DNA, 30 bp, Mus musculus
gctcgaagttcctacggggcaatggactac

SEQ ID NO: 24 - DNA, 27 bp, Mus musculus
cagcaatataacaactttccgtacacg

SEQ ID NO: 25 - protein, 16 aa, Homo sapiens
EVQVTMCIGACPSQFR

SEQ ID NO: 26 - protein, 21 aa, Homo sapiens
TDTGVSLQTYDDLLAKDCHCI